European Patent Application EP 4 553 502 A1, published May 14, 2025. Title: Cell surface antigen discovery method for novel antibody. Applicant: THE ASAN FOUNDATION. The sequence listing filed with the application follows.

SEQUENCE LISTING (20 sequences)

SEQ ID NO: 1 - DNA, 20 bp, synthetic construct
  misc_feature 1..20: note = artificial sequence
  source 1..20: mol_type = other DNA
tgtcaccacataattacctg

SEQ ID NO: 2 - DNA, 20 bp, synthetic construct
  misc_feature 1..20: note = artificial sequence
  source 1..20: mol_type = other DNA
gtggagcctcttacacccag

SEQ ID NO: 3 - DNA, 20 bp, synthetic construct
  misc_feature 1..20: note = artificial sequence
  source 1..20: mol_type = other DNA
gtctgcgtacttccagacca

SEQ ID NO: 4 - DNA, 20 bp, synthetic construct
  misc_feature 1..20: note = artificial sequence
  source 1..20: mol_type = other DNA
tcttgccggaatgtcagccg

SEQ ID NO: 5 - DNA, 20 bp, synthetic construct
  misc_feature 1..20: note = artificial sequence
  source 1..20: mol_type = other DNA
cctcattgccctcaacacag

SEQ ID NO: 6 - DNA, 20 bp, synthetic construct
  misc_feature 1..20: note = artificial sequence
  source 1..20: mol_type = other DNA
ctcttcttagaccatccagg

SEQ ID NO: 7 - DNA, 20 bp, synthetic construct
  misc_feature 1..20: note = artificial sequence
  source 1..20: mol_type = other DNA
catcacggttaacaatagct

SEQ ID NO: 8 - DNA, 20 bp, synthetic construct
  misc_feature 1..20: note = artificial sequence
  source 1..20: mol_type = other DNA
aagactcccattcgacaaca

SEQ ID NO: 9 - DNA, 20 bp, synthetic construct
  misc_feature 1..20: note = artificial sequence
  source 1..20: mol_type = other DNA
tgctacttcagacaaccaca

SEQ ID NO: 10 - DNA, 20 bp, synthetic construct
  misc_feature 1..20: note = artificial sequence
  source 1..20: mol_type = other DNA
tcgctacagcatctctcgga

SEQ ID NO: 11 - DNA, 20 bp, synthetic construct
  misc_feature 1..20: note = artificial sequence
  source 1..20: mol_type = other DNA
cgtggaatacacctgcaaag

SEQ ID NO: 12 - DNA, 20 bp, synthetic construct
  misc_feature 1..20: note = artificial sequence
  source 1..20: mol_type = other DNA
ctacagcatctctcggacgg

SEQ ID NO: 13 - DNA, 20 bp, synthetic construct
  misc_feature 1..20: note = artificial sequence
  source 1..20: mol_type = other DNA
tgacgtgtgcagtaatactg

SEQ ID NO: 14 - DNA, 20 bp, synthetic construct
  misc_feature 1..20: note = artificial sequence
  source 1..20: mol_type = other DNA
gcccgctgaggtcacgacca

SEQ ID NO: 15 - DNA, 20 bp, synthetic construct
  misc_feature 1..20: note = artificial sequence
  source 1..20: mol_type = other DNA
cgggctgttcccagtctcgg

SEQ ID NO: 16 - DNA, 20 bp, synthetic construct
  misc_feature 1..20: note = artificial sequence
  source 1..20: mol_type = other DNA
tgcagggactccagaacggg

SEQ ID NO: 17 - DNA, 20 bp, synthetic construct
  misc_feature 1..20: note = artificial sequence
  source 1..20: mol_type = other DNA
accagcacggagcctccccg

SEQ ID NO: 18 - DNA, 20 bp, synthetic construct
  misc_feature 1..20: note = artificial sequence
  source 1..20: mol_type = other DNA
gctcagttactcacagtaca

SEQ ID NO: 19 - RNA, 23 nt, synthetic construct
  misc_feature 1..23: note = artificial sequence
  source 1..23: mol_type = other RNA
ccggtatgagattgtcatcattt

SEQ ID NO: 20 - RNA, 23 nt, synthetic construct
  misc_feature 1..23: note = artificial sequence
  source 1..23: mol_type = other RNA
atgatgacaatctcataccggtt